European Patent Application EP 4 796 558 A1, published August 26, 2026. Title: 一种角蛋白CF3、制法和其药物组合物与用途. Applicant: 中国医学科学院药物研究所. The sequence listing filed with the application follows.

SEQUENCE LISTING (2 sequences)

SEQ ID NO: 1 - protein, 601 aa, unidentified
MSRQSSVSFRTGGSRSFSTASAVTPSVSRTSFTSVSRSGGGGGGFGRVSLGGACGVGGYGSRSLYNLGGSKRISISASGGGFRNRFGAGAGGGFGFGGGAGSGFGFGGGAGGGFGLGGGAGFGGGFGGPGFPVCPPGGIQEVTVNQSLLTPLNLQIDPAIQRVRTEEREQIKTLNNKFASFIDKVRFLEQQNKVLDTKWTLLQEQGTKTVRQNLEPLFEQYINNLRRQLDGILGERGRLDSELRNMQDLVEDFKNKYEDEINKRTTAENEFVMLKKDVDAAYMNKVELEAKVDALMDEINFMRMFFEAELSQMQTHISDTSVILSMDNNRSLDLDSIIAEVKAQYEEIANRSRTEAESWYQTKYEELQQTAGRHGDDLRNTKHEISEMNRMIQRLRAEIDNVKKQCANLQAAIADAEQRGELALKDARNKLAELEDALQKAKQDMARLLREYQELMNTKLALDVEIATYRKLLEGEECRLSHHVLPPFSAAVVTNTVSSAYGGGSGFGGGLGGGLGGGLGGGLGGGLGGGLGGGLGGGSSGGYYSSSSGGGGLSSGLSVGGSGFSASSGRGLGVGLGGGGGSSSSVKFVSTTSSSRKSFKS

SEQ ID NO: 2 - DNA, 1803 bp, unidentified
  source 1..1803: mol_type = other DNA
atgagccgccagagcagcgtgagctttcgtaccggtggtagccgctcatttagcaccgcgagcgcggtgaccccttcagtttcacgtactagctttaccagcgttagccgtagcggcggtggtggcggtggttttggccgtgttagcttaggtggtgcgtgtggcgtgggcggttatggttcacgtagcttatataatctgggcggcagcaaacgcattagcattagcgcgagcggcggcggctttcgcaatcgttttggtgcgggtgcgggtggtggatttggttttggtggtggtgcgggcagcggttttggctttggtggtggtgcaggtggcggttttggtttaggtggcggtgcaggctttggtggtggttttggtggtccgggttttccggtttgtccgccgggtggtattcaagaagtgaccgtgaatcagagcctgctgaccccgttaaacctgcagattgatccggcgattcagcgcgtgcgcaccgaagaacgtgaacagattaaaaccctgaacaacaaattcgcgagcttcatcgataaggtgcgctttctggaacagcagaacaaagtgctggataccaaatggaccctgctgcaggaacagggcaccaaaaccgtgcgccaaaacctggaaccgctgtttgaacagtatattaacaacctgcgccgccagctggatggcattctgggtgaacgtggtcgcttagatagcgaactgcgtaacatgcaggatctggtggaagattttaaaaacaagtacgaggacgagatcaacaagcgcaccaccgcggaaaacgaatttgtgatgctgaaaaaagacgtggacgcggcgtatatgaacaaagtggaactggaagcgaaagtggatgcgctgatggatgaaattaactttatgcgcatgtttttcgaggcggagctgagccagatgcagacccatattagcgataccagcgtgattctgagcatggataacaaccgcagcctggatctggatagcattattgcggaagtgaaagcgcagtatgaagaaattgcgaaccgcagccgcaccgaagcggaaagctggtatcaaaccaaatatgaagaactgcagcagaccgcgggccgccatggtgatgatttgcgtaataccaaacatgagattagcgagatgaaccgcatgatccagcgcctgcgcgcggaaattgataacgtgaaaaaacagtgcgcgaacctgcaggcggcgattgcggatgcagaacagcgtggtgaactggcgttaaaagatgcgcgcaataaactggcggaactggaagatgcgctgcagaaagcgaaacaggatatggcgcgcctgctgcgcgaatatcaggaactgatgaacaccaaactggcgctggatgtggaaattgcgacctatcgcaaactgctggaaggcgaagaatgccgcctgagccatcatgtgctgccgccttttagcgcggcggttgttaccaataccgtgagcagcgcgtatggcggcggttcaggttttggtggcggtttaggtggtggtttaggtggtggtttaggtggtggtttaggtggcggtctgggtggtggtttaggtggtggtttgggtggtggtagcagcggtggttattatagcagcagcagcggcggtggcggtctgtcatcaggtttaagcgttggtggcagcggttttagcgcgagcagcggccgtggtttaggtgttggtttaggcggtggcggtggcagcagcagctcagttaaatttgtgagcaccaccagcagcagccgcaaaagctttaaaagc